European Patent Application EP 4 653 449 A1, published November 26, 2025. Title: ブロック共重合体もしくはこれを含有する水分散液、接着剤、塗液、コーティング剤、又は成形体の製造方法. Applicant: Ｓｐｉｂｅｒ株式会社. The sequence listing filed with the application follows.

SEQUENCE LISTING (11 sequences)

SEQ ID NO: 1 - protein, 2375 aa, synthetic construct
  source 1..2375: note = PRT799
MHHHHHHSSGSSGPGQQGPYGPGASAAAAAGQNGPGSGQQGPGQSGQYGPGQQGPGQQGPGSSAAAAAGPGQYGPGQQGPSASAAAAAGPGSGQQGPGASGQYGPGQQGPGQQGPGSSAAAAAGQYGSGPGQQGPYGSAAAAAGPGSGQYGQGPYGPGASGPGQYGPGQQGPSASAAAAAGSGQQGPGQYGPYASAAAAAGQYGSGPGQQGPYGPGQSGSGQQGPGQQGPYASAAAAAGPGQQGPYGPGSSAAAAAGQYGYGPGQQGPYGPGASGQNGPGSGQYGPGQQGPGQSAAAAAGPGQQGPYGPGASAAAAAGQYGPGQQGPGQYGPGSSGPGQQGPYGPGSSAAAAAGQYGPGQQGPYGPGQSAAAAAGQYQQGPGQQGPYGPGASGPGQQGPYGPGASAAAAAGPGQYGPGQQGPSASAAAAAGQYGSGPGQYGPYGPGQSGPGSGQQGQGPYGPGASAAAAAGQYGPGQQGPYGPGQSAAAAAGPGSGQYGPGASGQNGPGSGQYGPGQQGPGQSAAAAAGQYQQGPGQQGPYGPGASAAAAAGQYGSGPGQQGPYGPGQSGSGQQGPGQQGPYASAAAAAGPGSGQQGPGASGQQGPYGPGASAAAAAGQNGPGSGQQGPGQSGQYGPGQQGPGQQGPGSSAAAAAGPGQYGPGQQGPSASAAAAAGPGSGQQGPGASGQYGPGQQGPGQQGPGSSAAAAAGQYGSGPGQQGPYGSAAAAAGPGSGQYGQGPYGPGASGPGQYGPGQQGPSASAAAAAGSGQQGPGQYGPYASAAAAAGQYGSGPGQQGPYGPGQSGSGQQGPGQQGPYASAAAAAGPGQQGPYGPGSSAAAAAGQYGYGPGQQGPYGPGASGQNGPGSGQYGPGQQGPGQSAAAAAGPGQQGPYGPGASAAAAAGQYGPGQQGPGQYGPGSSGPGQQGPYGPGSSAAAAAGQYGPGQQGPYGPGQSAAAAAGQYQQGPGQQGPYGPGASGPGQQGPYGPGASAAAAAGPGQYGPGQQGPSASAAAAAGQYGSGPGQYGPYGPGQSGPGSGQQGQGPYGPGASAAAAAGQYGPGQQGPYGPGQSAAAAAGPGSGQYGPGASGQNGPGSGQYGPGQQGPGQSAAAAAGQYQQGPGQQGPYGPGASAAAAAGQYGSGPGQQGPYGPGQSGSGQQGPGQQGPYASAAAAAGPGSGQQGPGASGQQGPYGPGASAAAAAGQNGPGSGQQGPGQSGQYGPGQQGPGQQGPGSSAAAAAGPGQYGPGQQGPSASAAAAAGPGSGQQGPGASGQYGPGQQGPGQQGPGSSAAAAAGQYGSGPGQQGPYGSAAAAAGPGSGQYGQGPYGPGASGPGQYGPGQQGPSASAAAAAGSGQQGPGQYGPYASAAAAAGQYGSGPGQQGPYGPGQSGSGQQGPGQQGPYASAAAAAGPGQQGPYGPGSSAAAAAGQYGYGPGQQGPYGPGASGQNGPGSGQYGPGQQGPGQSAAAAAGPGQQGPYGPGASAAAAAGQYGPGQQGPGQYGPGSSGPGQQGPYGPGSSAAAAAGQYGPGQQGPYGPGQSAAAAAGQYQQGPGQQGPYGPGASGPGQQGPYGPGASAAAAAGPGQYGPGQQGPSASAAAAAGQYGSGPGQYGPYGPGQSGPGSGQQGQGPYGPGASAAAAAGQYGPGQQGPYGPGQSAAAAAGPGSGQYGPGASGQNGPGSGQYGPGQQGPGQSAAAAAGQYQQGPGQQGPYGPGASAAAAAGQYGSGPGQQGPYGPGQSGSGQQGPGQQGPYASAAAAAGPGSGQQGPGASGQQGPYGPGASAAAAAGQNGPGSGQQGPGQSGQYGPGQQGPGQQGPGSSAAAAAGPGQYGPGQQGPSASAAAAAGPGSGQQGPGASGQYGPGQQGPGQQGPGSSAAAAAGQYGSGPGQQGPYGSAAAAAGPGSGQYGQGPYGPGASGPGQYGPGQQGPSASAAAAAGSGQQGPGQYGPYASAAAAAGQYGSGPGQQGPYGPGQSGSGQQGPGQQGPYASAAAAAGPGQQGPYGPGSSAAAAAGQYGYGPGQQGPYGPGASGQNGPGSGQYGPGQQGPGQSAAAAAGPGQQGPYGPGASAAAAAGQYGPGQQGPGQYGPGSSGPGQQGPYGPGSSAAAAAGQYGPGQQGPYGPGQSAAAAAGQYQQGPGQQGPYGPGASGPGQQGPYGPGASAAAAAGPGQYGPGQQGPSASAAAAAGQYGSGPGQYGPYGPGQSGPGSGQQGQGPYGPGASAAAAAGQYGPGQQGPYGPGQSAAAAAGPGSGQYGPGASGQNGPGSGQYGPGQQGPGQSAAAAAGQYQQGPGQQGPYGPGASAAAAAGQYGSGPGQQGPYGPGQSGSGQQGPGQQGPYASAAAAAGPGSGQQGSSVDKLAAALEHHHHHH

SEQ ID NO: 2 - protein, 1190 aa, synthetic construct
  source 1..1190: note = PRT966
MHHHHHHSSGSSGPGVFGPYGPGASAAAAAGINGPGSGVFGPGISGIYGPGVFGPGVFGPGSSAAAAAGPGIYGPGVFGPSASAAAAAGPGSGVFGPGASGIYGPGVFGPGVFGPGSSAAAAAGIYGSGPGVFGPYGSAAAAAGPGSGIYGIGPYGPGASGPGIYGPGVFGPSASAAAAAGSGVFGPGIYGPYASAAAAAGIYGSGPGVFGPYGPGISGSGVFGPGVFGPYASAAAAAGPGVFGPYGPGSSAAAAAGIYGYGPGVFGPYGPGASGINGPGSGIYGPGVFGPGISAAAAAGPGVFGPYGPGASAAAAAGIYGPGVFGPGIYGPGSSGPGVFGPYGPGSSAAAAAGIYGPGVFGPYGPGISAAAAAGIYVFGPGVFGPYGPGASGPGVFGPYGPGASAAAAAGPGIYGPGVFGPSASAAAAAGIYGSGPGIYGPYGPGISGPGSGVFGIGPYGPGASAAAAAGIYGPGVFGPYGPGISAAAAAGPGSGIYGPGASGINGPGSGIYGPGVFGPGISAAAAAGIYVFGPGVFGPYGPGASAAAAAGIYGSGPGVFGPYGPGISGSGVFGPGVFGPYASAAAAAGPGSGVFGPGASGPGVFGPYGPGASAAAAAGINGPGSGVFGPGISGIYGPGVFGPGVFGPGSSAAAAAGPGIYGPGVFGPSASAAAAAGPGSGVFGPGASGIYGPGVFGPGVFGPGSSAAAAAGIYGSGPGVFGPYGSAAAAAGPGSGIYGIGPYGPGASGPGIYGPGVFGPSASAAAAAGSGVFGPGIYGPYASAAAAAGIYGSGPGVFGPYGPGISGSGVFGPGVFGPYASAAAAAGPGVFGPYGPGSSAAAAAGIYGYGPGVFGPYGPGASGINGPGSGIYGPGVFGPGISAAAAAGPGVFGPYGPGASAAAAAGIYGPGVFGPGIYGPGSSGPGVFGPYGPGSSAAAAAGIYGPGVFGPYGPGISAAAAAGIYVFGPGVFGPYGPGASGPGVFGPYGPGASAAAAAGPGIYGPGVFGPSASAAAAAGIYGSGPGIYGPYGPGISGPGSGVFGIGPYGPGASAAAAAGIYGPGVFGPYGPGISAAAAAGPGSGIYGPGASGINGPGSGIYGPGVFGPGISAAAAAGIYVFGPGVFGPYGPGASAAAAAGIYGSGPGVFGPYGPGISGSGVFGPGVFGPYASAAAAAGPGSGVFGPGAS

SEQ ID NO: 3 - protein, 601 aa, synthetic construct
  source 1..601: note = PRT918
MHHHHHHSSGSSGPGVFGPYGPGASAAAAAGINGPGSGVFGPGISGIYGPGVFGPGVFGPGSSAAAAAGPGIYGPGVFGPSASAAAAAGPGSGVFGPGASGIYGPGVFGPGVFGPGSSAAAAAGIYGSGPGVFGPYGSAAAAAGPGSGIYGIGPYGPGASGPGIYGPGVFGPSASAAAAAGSGVFGPGIYGPYASAAAAAGIYGSGPGVFGPYGPGISGSGVFGPGVFGPYASAAAAAGPGVFGPYGPGSSAAAAAGIYGYGPGVFGPYGPGASGINGPGSGIYGPGVFGPGISAAAAAGPGVFGPYGPGASAAAAAGIYGPGVFGPGIYGPGSSGPGVFGPYGPGSSAAAAAGIYGPGVFGPYGPGISAAAAAGIYVFGPGVFGPYGPGASGPGVFGPYGPGASAAAAAGPGIYGPGVFGPSASAAAAAGIYGSGPGIYGPYGPGISGPGSGVFGIGPYGPGASAAAAAGIYGPGVFGPYGPGISAAAAAGPGSGIYGPGASGINGPGSGIYGPGVFGPGISAAAAAGIYVFGPGVFGPYGPGASAAAAAGIYGSGPGVFGPYGPGISGSGVFGPGVFGPYASAAAAAGPGSGVFGPGAS

SEQ ID NO: 4 - protein, 608 aa, synthetic construct
  source 1..608: note = PRT313
MHHHHHHSSGSSGPGGQGPYGPGASAAAAAGGNGPGSGQQGPGGSAAAAAGGYGPGGQGPGQQGPGSSAAAAAGPGGYGPGGQGPSASAAAAAGPGSGQQGPGASAAAAAGGYGPGGQGPGQQGPGSSAAAAAGGYGSGPGQQGPYGSAAAAAGPGSGGYGQGPYGPGASAAAAAGPGGYGPGGQGPSASAAAAAGSGQQGPGGYGPYASAAAAAGGYGSGPGQQGPYGPGGSAAAAAGSGQQGPGQQGPYASAAAAAGPGGQGPYGPGSSAAAAAGGYGYGPGGQGPYGPGASAAAAAGGNGPGSGGYGPGQQGPGGSAAAAAGPGGQGPYGPGASAAAAAGGYGPGGQGPGGYGPGSSAAAAAGPGGQGPYGPGSSAAAAAGGYGPGQQGPYGPGGSAAAAAGGYQQGPGGQGPYGPGASAAAAAGPGGQGPYGPGASAAAAAGPGGYGPGGQGPSASAAAAAGGYGSGPGGYGPYGPGGSAAAAAGPGSGQQGQGPYGPGASAAAAAGGYGPGQQGPYGPGGSAAAAAGPGSGGYGPGASAAAAAGGNGPGSGGYGPGQQGPGGSAAAAAGGYQQGPGGQGPYGPGASAAAAAGPGSGQQGPGAS

SEQ ID NO: 5 - protein, 603 aa, synthetic construct
  source 1..603: note = PRT1000
MHHHHHHSSGSSCGPGVFGPYGPGASAAAAAGINGPGSGVFGPGISGIYGPGVFGPGVFGPGSSAAAAAGPGIYGPGVFGPSASAAAAAGPGSGVFGPGASGIYGPGVFGPGVFGPGSSAAAAAGIYGSGPGVFGPYGSAAAAAGPGSGIYGIGPYGPGASGPGIYGPGVFGPSASAAAAAGSGVFGPGIYGPYASAAAAAGIYGSGPGVFGPYGPGISGSGVFGPGVFGPYASAAAAAGPGVFGPYGPGSSAAAAAGIYGYGPGVFGPYGPGASGINGPGSGIYGPGVFGPGISAAAAAGPGVFGPYGPGASAAAAAGIYGPGVFGPGIYGPGSSGPGVFGPYGPGSSAAAAAGIYGPGVFGPYGPGISAAAAAGIYVFGPGVFGPYGPGASGPGVFGPYGPGASAAAAAGPGIYGPGVFGPSASAAAAAGIYGSGPGIYGPYGPGISGPGSGVFGIGPYGPGASAAAAAGIYGPGVFGPYGPGISAAAAAGPGSGIYGPGASGINGPGSGIYGPGVFGPGISAAAAAGIYVFGPGVFGPYGPGASAAAAAGIYGSGPGVFGPYGPGISGSGVFGPGVFGPYASAAAAAGPGCSGVFGPGAS

SEQ ID NO: 6 - protein, 605 aa, synthetic construct
  source 1..605: note = PRT1001
MHHHHHHSSGSSCGPGVFGPYGPGASAAAAAGINGPGSGVFGPGISCGIYGPGVFGPGVFGPGSSAAAAAGPGIYGPGVFGPSASAAAAAGPGSGVFGPGASGIYGPGVFGPGVFGPGSSAAAAAGIYGSGPGVFGPYGSAAAAAGPGSGIYGIGPYGPGASGPGIYGPGVFGPSASAAAAAGSGVFGPGIYGPYASAAAAAGIYGSGPGVFGPYGPGISGSGVFGPGVFGPYASAAAAAGPGVFGPYGPGSSAAAAAGIYGYGPGVFGPYGPGASGINGPGSGIYGPGVFGPGISAAAAAGPGVFGPYGPGASAAAAAGIYGPGVFGPGIYGPGSSGPGVFGPYGPGSSAAAAAGIYGPGVFGPYGPGISAAAAAGIYVFGPGVFGPYGPGASGPGVFGPYGPGASAAAAAGPGIYGPGVFGPSASAAAAAGIYGSGPGIYGPYGPGISGPGSGVFGIGPYGPGASAAAAAGIYGPGVFGPYGPGISAAAAAGPGSGIYGPGASGINGPGSGIYGPGVFGPGISAAAAAGIYVFGPGVFGPYGPGASAAAAAGIYGSGPGVFGPYGPGISGCSGVFGPGVFGPYASAAAAAGPGCSGVFGPGAS

SEQ ID NO: 7 - protein, 1188 aa, synthetic construct
  source 1..1188: note = PRT587
MHHHHHHSSGSSGPGQQGPYGPGASAAAAAGQNGPGSGQQGPGQSGQYGPGQQGPGQQGPGSSAAAAAGPGQYGPGQQGPSASAAAAAGPGSGQQGPGASGQYGPGQQGPGQQGPGSSAAAAAGQYGSGPGQQGPYGSAAAAAGPGSGQYGQGPYGPGASGPGQYGPGQQGPSASAAAAAGSGQQGPGQYGPYASAAAAAGQYGSGPGQQGPYGPGQSGSGQQGPGQQGPYASAAAAAGPGQQGPYGPGSSAAAAAGQYGYGPGQQGPYGPGASGQNGPGSGQYGPGQQGPGQSAAAAAGPGQQGPYGPGASAAAAAGQYGPGQQGPGQYGPGSSGPGQQGPYGPGSSAAAAAGQYGPGQQGPYGPGQSAAAAAGQYQQGPGQQGPYGPGASGPGQQGPYGPGASAAAAAGPGQYGPGQQGPSASAAAAAGQYGSGPGQYGPYGPGQSGPGSGQQGQGPYGPGASAAAAAGQYGPGQQGPYGPGQSAAAAAGPGSGQYGPGASGQNGPGSGQYGPGQQGPGQSAAAAAGQYQQGPGQQGPYGPGASAAAAAGQYGSGPGQQGPYGPGQSGSGQQGPGQQGPYASAAAAAGPGSGQQGPGASGQQGPYGPGASAAAAAGQNGPGSGQQGPGQSGQYGPGQQGPGQQGPGSSAAAAAGPGQYGPGQQGPSASAAAAAGPGSGQQGPGASGQYGPGQQGPGQQGPGSSAAAAAGQYGSGPGQQGPYGSAAAAAGPGSGQYGQGPYGPGASGPGQYGPGQQGPSASAAAAAGSGQQGPGQYGPYASAAAAAGQYGSGPGQQGPYGPGQSGSGQQGPGQQGPYASAAAAAGPGQQGPYGPGSSAAAAAGQYGYGPGQQGPYGPGASGQNGPGSGQYGPGQQGPGQSAAAAAGPGQQGPYGPGASAAAAAGQYGPGQQGPGQYGPGSSGPGQQGPYGPGSSAAAAAGQYGPGQQGPYGPGQSAAAAAGQYQQGPGQQGPYGPGASGPGQQGPYGPGASAAAAAGPGQYGPGQQGPSASAAAAAGQYGSGPGQYGPYGPGQSGPGSGQQGQGPYGPGASAAAAAGQYGPGQQGPYGPGQSAAAAAGPGSGQYGPGASGQNGPGSGQYGPGQQGPGQSAAAAAGQYQQGPGQQGPYGPGASAAAAAGQYGSGPGQQGPYGPGQSGSGQQGPGQQGPYASAAAAAGPGSGQQGPGAS

SEQ ID NO: 8 - protein, 313 aa, synthetic construct
  source 1..313: note = PRT2662
MHHHHHHSSGSSCGPGVFGPYGPGASAAAAAGINGPGSGVFGPGISGIYGPGVFGPGVFGPGSSAAAAAGPGIYGPGVFGPSASAAAAAGPGSGVFGPGASGIYGPGVFGPGVFGPGSSAAAAAGIYGSGPGVFGPYGSAAAAAGPGSGIYGIGPYGPGASGPGIYGPGVFGPSASAAAAAGSGVFGPGIYGPYASAAAAAGIYGSGPGVFGPYGPGISGSGVFGPGVFGPYASAAAAAGPGVFGPYGPGSSAAAAAGIYGYGPGVFGPYGPGASGINGPGSGIYGPGVFGPGISAAAAAGPGCSGVFGPGAS

SEQ ID NO: 9 - protein, 24 aa, synthetic construct
  source 1..24: note = His tag and start codon
MHHHHHHHHHHSSGSSLEVLFQGP

SEQ ID NO: 10 - protein, 110 aa, synthetic construct
MHHHHHHSSGSSCGPGVFGPYGPGASAAAAAGINGPGSGVFGPGISGIYGPGVFGPGVFGPGSSAAAAAGPGIYGPGVFGPSASAAAAAGPGCSGVFGPGASGFILGFIL

SEQ ID NO: 11 - protein, 120 aa, synthetic construct
MHHHHHHKGFILGFILSSGSSCGPGVFGPYGPGASAAAAAGINGPGSGVFGPGISGIYGPGVFGPGVFGPGSSAAAAAGPGIYGPGVFGPSASAAAAAGPGSGVFGPGKASGFILGFILC